European Patent Application EP 4 169 940 A1, published April 26, 2023. Title: Low molecular weight antibody with reduced immunogenicity. Applicant: Kyoto University. The sequence listing filed with the application follows.

SEQUENCE LISTING (74 sequences)

SEQ ID NO: 1 - protein, 25 aa, Camelus dromedarius
QVQLVESGGALVQPGGSLRLSCAAS

SEQ ID NO: 2 - protein, 14 aa, Camelus dromedarius
WYRQAPGKEREWVA

SEQ ID NO: 3 - protein, 38 aa, Camelus dromedarius
YEDSVKGRFTISRDDARNTVYLQMNSLKPEDTAVYYCN

SEQ ID NO: 4 - protein, 11 aa, Camelus dromedarius
WGQGTQVTVSS

SEQ ID NO: 5 - protein, 25 aa, Lama glama
QVQLQESGGGLVQAGGSLRLSCAAA

SEQ ID NO: 6 - protein, 14 aa, Lama glama
WFRQAPGKEREFVG

SEQ ID NO: 7 - protein, 38 aa, Lama glama
YADSVKGRFIISRDNAKNTVYLQMNSLKPEDTAVYYCA

SEQ ID NO: 8 - protein, 11 aa, Lama glama
WGQGTQVTVSS

SEQ ID NO: 9 - protein, 25 aa, Vicugna pacos
QVQLQESGGGLVQPGGSLRLSCAAS

SEQ ID NO: 10 - protein, 14 aa, Vicugna pacos
WYRQAPGKERELVA

SEQ ID NO: 11 - protein, 36 aa, Vicugna pacos
DSVKGRYTISRDYAKNTVYLQMNSLKPEDTALYYCN

SEQ ID NO: 12 - protein, 11 aa, Vicugna pacos
WGQGTQVTVSS

SEQ ID NO: 13 - protein, 25 aa, Vicugna pacos
QVQLQESGGGLVQPGGSLRLSCAAS

SEQ ID NO: 14 - protein, 14 aa, Vicugna pacos
WFRQAPGKEREFVA

SEQ ID NO: 15 - protein, 38 aa, Vicugna pacos
YADSVKGRFTISRDNAKNTVYLQMNSLKPEDTAVYYCA

SEQ ID NO: 16 - protein, 11 aa, Vicugna pacos
WGQGTQVTVSS

SEQ ID NO: 17 - protein, 25 aa, Camelus dromedarius
QVQLVESGGGSVQAGGSLRLSCTAS

SEQ ID NO: 18 - protein, 14 aa, Camelus dromedarius
WYHQAPGNECELVS

SEQ ID NO: 19 - protein, 38 aa, Camelus dromedarius
YADSVKGRFTISRDNAKNTVYLQMNSLKPEDTAMYYCA

SEQ ID NO: 20 - protein, 11 aa, Camelus dromedarius
WGQGTQVTVSS

SEQ ID NO: 21 - protein, 128 aa, Camelus dromedarius
QVQLQESGGGSVQTGGSLRLSCAASEYTQSSACMGWFRQAPGKEREGVAGISRFFGTAYYADSVKGRFTISQDKAKNTVYLQMNSLKPEDTAIYYCAAGQGCLTTIQALGGAYGYNAWGQGTQVTVSS

SEQ ID NO: 22 - protein, 128 aa, Camelidae
QVQLQESGGGLVQPGGSLRLSCAASGKMSSRRCMAWFRQAPGKERERVAKLLTTSGSTYLADSVKGRFTISQNNAKSTVYLQMNSLKPEDTAMYYCAADSFEDPTCTLVTSSGAFQYWGQGTQVTVSS

SEQ ID NO: 23 - protein, 125 aa, Lama glama
QVQLQESGGGLVQPGGSLRLSCAASGFTLDYYYIGWFRQAPGKEREGVSCISSSHGSTYYADSVKGRFTISRDNAKNTVYLQMNSLKPEDTAVYYCATVAVAHFRGCGVDGMDYWGKGTQVTVSS

SEQ ID NO: 24 - protein, 115 aa, Lama glama
QVQLVESGGALVQPGGSLRLSCAASGFPVNRYSMRWFRQAPGKEREWVAGMSSAGDRSSYEDSVKGRFTISRDDARNTVYLQMNSLKPEDTAVYYCNVNVGFEYWGQGTQVTVSS

SEQ ID NO: 25 - protein, 128 aa, Artificial Sequence
  Humanized VHH (human-lama)
EVQLVESGGGLVQPGGSLRLSCAASGRTFSYNPMGWFRQAPGKGRELVAAISRTGGSTYYPDSVEGRFTISRDNAKRMVYLQMNSLRAEDTAVYYCAAAGVRAEDGRVRTLPSEYTFWGQGTQVTVSS

SEQ ID NO: 26 - protein, 125 aa, Lama glama
QVQLQESGGGLVQAGGSLRLSCAASGRTFSEYAMGWFRQAPGKEREFVATISWSGGSTYYTDSVKGRFTISRDNAKNTVYLQMNSLKPDDTAVYYCAAAGLGTVVSEWDYDYDYWGQGTQVTVSS

SEQ ID NO: 27 - protein, 120 aa, Lama glama
QVQLQESGGGSVQAGGSLRLSCVASGSIFSINAMDWYRQAPGKQRELVAGITSGGSTNYGDFVKGRFTISRDNAKNTVYLQMDSLKPEDTAVYYCAAEVGGWGPPRPDYWGHGTQVTVSS

SEQ ID NO: 28 - protein, 123 aa, Camelus dromedarius
QVQLQESGGGSVQAGGSLRLSCAASGYTLSTYCMGWFRQAPGKEHEGAAFINSGGGNEYYADSVKGRFTISQDNAKNTVLLQMNSLKPEDTAIYYCAAGRYCIGGYPGGGTYWGQGTQVTVSS

SEQ ID NO: 29 - protein, 117 aa, Camelus dromedarius
QVQLQESGGGSVQAGGSLRLSCTASGFGVDGTDMGWYRQAPGNECELVSSISSIGIGYYSESVKGRFTISRDNAKNTVYLQMNSLRPDDTAVYYCGRRWIGYRCGNWGRGTQVTVSS

SEQ ID NO: 30 - protein, 118 aa, Camelus dromedarius
EVQLVESGGGLVQAGGSLRLSCAASGITFSINTMGWYRQAPGKQRELVALISSIGDTYYADSVKGRFTISRDNAKNTVYLQMNSLKPEDTAVYYCKRFRTAAQGTDYWGQGTQVTVSS

SEQ ID NO: 31 - protein, 122 aa, Lama glama
QVQLQESGGGLVQAGGSLRLSCAAAGRNLRMYRMGWFRQAPGKEREFVGTMVWSSDTIYYADSVKGRFIISRDNAKNTVYLQMNSLKPEDTAVYYCAAGAGWAGTMTDYNYWGQGTQVTVSS

SEQ ID NO: 32 - protein, 127 aa, Lama glama
QVQLQESGGGLVQAGGSLRLSCAASGRTFTSFAMGWFRQAPGKEREFVASISRSGTLTRYADSAKGRFTISVDNAKNTVSLQMDNLNPDDTAVYYCAADLHRPYGPGTQRSDEYDSWGQGTQVTVSS

SEQ ID NO: 33 - protein, 127 aa, Lama glama
QVQLQESGGGLVQPGGSLRLSCAASGRTFSNYRMGWFRQAPGKEREFVATISQSGAATAYADSVKGRFTFSRDNAKNLLYLEMLSLEPEDTAVYYCAASSRVFYTEVLQTTTGYDYWGQGTQVTVSS

SEQ ID NO: 34 - protein, 125 aa, Lama glama
QVQLQESGGGLVQAGGSLRLSCAASGRTFSNDHMGWFRKAPGKEREFVAAITPGTEKTYYADSVKGRFAFSRDNAKNTVYLQMNSLKPEDTAVYYCVATPYYRGSYYAASTYTYWGQGTQVTVSS

SEQ ID NO: 35 - protein, 117 aa, Vicugna pacos
QVQLAESGGGLVQPGGSLRLSCSASGGVFIIYNMGWYRQAPGKQRELVASIDSYSGSITNYADSVKGRFTISRDNVEKRVYLEMNNLKPEDTAVYYCNANLRTNNYWGQGTQVTVSS

SEQ ID NO: 36 - protein, 118 aa, Vicugna pacos
QVQLQESGGGLVQPGGSLRLSCAASGSITSTNAMGWYRQAPGKERELVAQITNYGASNYGDSVKGRYTISRDYAKNTVYLQMNSLKPEDTALYYCNVREYRFEVADYWGQGTQVTVSS

SEQ ID NO: 37 - protein, 130 aa, Vicugna pacos
QVQLQESGGGLVQPGGSLRLSCAASGFTFDYYAVGWFRHAPGKEREGVSCISGGSTNYADSVKGRFTISRDNAKNTVYLQMNSLKPEDTAIYYCAAIKRGFCTSWGGEVPAPKSADYDYWGQGTQVTVSS

SEQ ID NO: 38 - protein, 122 aa, Vicugna pacos
QVQLQESGGGLVQPGGSLRLSCAASGFTFSRYPMNWVRQAPGKGLEWVAAINSSGEATLYADSVKGRFTISRDNAKNTLYLQMTGLKPEDTAVYYCADDGKLLPQSTTTWYRGQGTQVTVSS

SEQ ID NO: 39 - protein, 124 aa, Vicugna pacos
QVQLQESGGGVVQPGGSLTLSCTRTGFTASTNAYGWYRQGPGKKCEWVSYMTIPSGRTTYADAVKGRFAMSRDKAKSTVLLQMNSLKPEDTAVYYCGDVPFSTLPAMCTNDGPWGQGTQVTVSS

SEQ ID NO: 40 - protein, 124 aa, Vicugna pacos
QVQLQESGGGVVQPGGSLTLSCTRTGLTPSTGAYGWYRQAPGKKCELVSYITIPSGRTTYTDSVKGRFAISRDKAKNTVFLQMNSLKPEDTALYYCGDVPYSTIQAMCTDDGPWGQGTQVTVSS

SEQ ID NO: 41 - protein, 124 aa, Vicugna pacos
QVQLQESGGGVVQPGGSLTLSCTRTGLTASTNAYGWYRQAPGKKCELVSYITIPSGRTTYADSVKGRFAISRDKAKNTVFLQMNSLKPEDTALYYCGDVPYSTIQAMCTDDGPWGQGTQVTVSS

SEQ ID NO: 42 - protein, 114 aa, Vicugna pacos
QVQLQESGGGLVQSGGSLRLSCRASGFTFSHYPMSWYRQAPGKKRELVAGIYTDGSTNYADSVKGRFTISRDNAKNTVYLQMSSLKPEDTAVYYCRRSMVSVYWGQGTQVTVSS

SEQ ID NO: 43 - protein, 120 aa, Vicugna pacos
QVQLQESGGGLVQPGGSLRLSCAASGRTFSYYTMAWFRQAPGKEREFVASISWSGGITYYADSVKGRFTISRDNAKNTVYLQMNSLKPEDTAVYYCAARKEPGSAYFGSWGQGTQVTVSS

SEQ ID NO: 44 - protein, 124 aa, Vicugna pacos
QVQLQESGGGVVQPGGSLTLSCTRTGFTASTNAYGWYRQAPGKKCELVSYITIPSGRTTYADAVKGRFAISRDKAKNTVFLQMNSLKPEDTAVYYCGDVPFSTLPAMCTNDGPWGQGTQVTVSS

SEQ ID NO: 45 - protein, 124 aa, Vicugna pacos
QVQLQESGGGVVQPGGSLTLSCTRTGFTASTNAYGWYRQGPGKKCEWVSYMTIPSGRTTYADAVKGRFAMSRDKAKSTVFLQMNSLKPEDTAVYYCGDVPFSTLPAMCTNDGPWGQGTQVTVSS

SEQ ID NO: 46 - protein, 126 aa, Camelus dromedarius
QVQLQESGGGLVQPGGSLRLSCAASGYPYGYTFSSYCMRWFRQAPGKDREGVARFERNGLTTYYDDSVKGRFTISQDNVKNTVYLQMNSLKPEDTATYYCAAAPKQLRTCGDYNYWGQGTQVTVSS

SEQ ID NO: 47 - protein, 131 aa, Camelus dromedarius
QVQLQESGGGSVQVGGSLRVACAASGDTFSGYLAAWFRQAPGKGREGVAAINSKRHTTSYADSVKGRFTISKDNADNIMYLEMNSLKPEDTAIYYCAAADAIGLAEYWSTPTLSAARYKYWGQGTQVTVSS

SEQ ID NO: 48 - protein, 129 aa, Camelus dromedarius
DVQLQESGGGSVQAGGSLRLSCAASPYFSLRSCVAWFRQAPGKEREGVAAIFTSTGSTYYADSVKGRFTISQDNANTVSLQMNSLKPEDAAMYYCAIEGRPMIGGPSCSMGSPNSYTYWGQGTQVTVSS

SEQ ID NO: 49 - protein, 127 aa, Camelus dromedarius
DVQLQESGGGSVQAGGSLRLSCSVSGYTFSMLAMAWFRQAPGKEREWVAVISPGSGFTYYDDSVKGRFTISRDNAKNTVYLQMNRLKSEDTAMYYCSAGLWSEGISNVRAPDGYKYWGQGTQVTVSS

SEQ ID NO: 50 - protein, 116 aa, Camelus dromedarius
QVQLQESGGGLVQAGGSLRLSCATSGSIFSIISMGWYRQAPGKQRELVALVFRGGSTVYADSVKGRFTISGDIAKSTVYLQMDSLKPEDTAVYYCNAKPIGTAQYWGQGTQVTVSS

SEQ ID NO: 51 - protein, 125 aa, Camelus dromedarius
QVQLVESGGGSVQAGGSLRLSCTASGFTFDDSDMGWYHQAPGNECELVSAIFSDGSTYYADSVKGRFTISRDNAKNTVYLQMNSLKPEDTAMYYCAAATTTVASPPVRHVCNGYWGQGTQVTVSS

SEQ ID NO: 52 - protein, 122 aa, Camelus dromedarius
  MOD_RES (116)..(122): lysine with His-tag
QVQLVESGGALVQPGGSLRLSCAASGFPVNRYSMRWYRQAPGKEREWVAGMSSAGDRSSYEDSVKGRFTISRDDARNTVYLQMNSLKPEDTAVYYCNVNVGFEYWGQGTQVTVSSKHHHHHH

SEQ ID NO: 53 - protein, 126 aa, Camelidae
  MOD_RES (121)..(126): His tag
  MOD_RES (121)..(126): His-tag
EVQLVESGGGLVQAGGSLRLSCATSGITFMRYALGWYRQSPGKQREMVASINSGGTTNYADSVKGRFTISRDNAKNTVYLQMNSLKPEDTAVYYCNARWVKPQFIDNNYWGQGTQVTVSSHHHHHH

SEQ ID NO: 54 - protein, 128 aa, Artificial Sequence; identical to SEQ ID NO: 25
  Humanized VHH (human-lama)

SEQ ID NO: 55 - protein, 21 aa, Artificial Sequence
  Synthetic peptide L-1/D-1
QVQLVESGGALVQPGGSLRLS

SEQ ID NO: 56 - protein, 32 aa, Artificial Sequence
  Syntheic peptide L-2/D-2
CAASGFPVNRYSMRWYRQAPGKEREWVAGMSS

SEQ ID NO: 57 - protein, 42 aa, Artificial Sequence
  Synthetic peptide L-3/D-3
CGDRSSYEDSVKGRFTISRDDARNTVYLQMNSLKPEDTAVYY

SEQ ID NO: 58 - protein, 27 aa, Artificial Sequence
  Synthetic peptide L-4/D-4
CNVNVGFEYWGQGTQVTVSSKHHHHHH

SEQ ID NO: 59 - protein, 74 aa, Artificial Sequence
  Synthetic peptide L-5/D-5
CAASGFPVNRYSMRWYRQAPGKEREWVAGMSSCGDRSSYEDSVKGRFTISRDDARNTVYLQMNSLKPEDTAVYY

SEQ ID NO: 60 - protein, 74 aa, Artificial Sequence
  Synthetic peptide L-6/D-6
CAASGFPVNRYSMRWYRQAPGKEREWVAGMSSAGDRSSYEDSVKGRFTISRDDARNTVYLQMNSLKPEDTAVYY

SEQ ID NO: 61 - protein, 74 aa, Artificial Sequence; identical to SEQ ID NO: 60
  Synthetic peptide L-7/D-7

SEQ ID NO: 62 - protein, 95 aa, Artificial Sequence
  Synthetic peptide L-8/D-8
QVQLVESGGALVQPGGSLRLSCAASGFPVNRYSMRWYRQAPGKEREWVAGMSSAGDRSSYEDSVKGRFTISRDDARNTVYLQMNSLKPEDTAVYY

SEQ ID NO: 63 - protein, 95 aa, Artificial Sequence; identical to SEQ ID NO: 62
  Synthetic peptide L-9/D-9

SEQ ID NO: 64 - protein, 122 aa, Artificial Sequence; identical to SEQ ID NO: 52
  Synthetic peptide L-10/D-10

SEQ ID NO: 65 - protein, 21 aa, Artificial Sequence
  Synthetic peptide L-11/D-11
EVQLVESGGGLVQPGGSLRLS

SEQ ID NO: 66 - protein, 28 aa, Artificial Sequence
  Synthetic peptide L-12/D-12
CAASGRTFSYNPMGWFRQAPGKGRELVA

SEQ ID NO: 67 - protein, 46 aa, Artificial Sequence
  Synthetic peptide L-13/D-13
CISRTGGSTYYPDSVEGRFTISRDNAKRMVYLQMNSLRAEDTAVYY

SEQ ID NO: 68 - protein, 33 aa, Artificial Sequence
  Synthetic peptide L-14/D-14
CAAAGVRAEDGRVRTLPSEYTFWGQGTQVTVSS

SEQ ID NO: 69 - protein, 74 aa, Artificial Sequence
  Synthetic peptide L-15/D-15
CAASGRTFSYNPMGWFRQAPGKGRELVACISRTGGSTYYPDSVEGRFTISRDNAKRMVYLQMNSLRAEDTAVYY

SEQ ID NO: 70 - protein, 74 aa, Artificial Sequence
  Synthetic peptide L-16/D-16
CAASGRTFSYNPMGWFRQAPGKGRELVAAISRTGGSTYYPDSVEGRFTISRDNAKRMVYLQMNSLRAEDTAVYY

SEQ ID NO: 71 - protein, 74 aa, Artificial Sequence; identical to SEQ ID NO: 70
  Synthetic peptide L-17/D-17

SEQ ID NO: 72 - protein, 95 aa, Artificial Sequence
  Synthetic peptide L-18/D-18
EVQLVESGGGLVQPGGSLRLSCAASGRTFSYNPMGWFRQAPGKGRELVAAISRTGGSTYYPDSVEGRFTISRDNAKRMVYLQMNSLRAEDTAVYY

SEQ ID NO: 73 - protein, 95 aa, Artificial Sequence; identical to SEQ ID NO: 72
  Synthetic peptide L-19/D-19

SEQ ID NO: 74 - protein, 128 aa, Artificial Sequence; identical to SEQ ID NO: 25
  Synthetic peptide L-20/D-20